European Patent Application EP 4 534 662 A1, published April 9, 2025. Title: Novel variant of 5-dehydro-2-deooxygluconokinase and method for producing 5'-inosinic acid using the same. Applicant: DAESANG CORPORATION. The sequence listing filed with the application follows.

SEQUENCE LISTING (9 sequences)

SEQ ID NO: 1 - DNA, 957 bp, synthetic construct
  source 1..957: mol_type = other DNA
atggcgtatttaactagcgctcacgaagttctggccatcggcaggcttggcgtggatatctatccactacagtccggcgttgggctagaagaggtatcttctttcggcaaatacctaggcggatccgcagcaaatgtctctgttgcagccgcacggcacgggcacaattccgcactgctatcacgagtaggcaatgacccactgggtaagtacctgctcaatgagctggaaaggctcggggtagataatcagtacgtcgctactgatccgacttataaaaccccgctgactttgtgcgaaattttcccaccagatgatttcccgctgtacttctaccgcgagcccaaagctccggatatgtgcatcgagtcctctgacgtcaacctcgaagatgtccgcgatgcagaaatcttgtggtttaccctgaccggtttaaacgaagagccaagccgcggcgcacatcaggaaatcctgaacacccgcgcccggcgcaagcacaccatcttggacttggactaccgcgacatgttctggaattccaagcaggaagcaacagagcaggcacagtgggcactcgagcatgccaccgttgcggtcggtaacaaggaagaatgcgaggtcgccatcggcgaaaccgaaccagaacgcgccggcaaggcgttgttggaacatggcgtgaagttggccatcgttaagcaaggccccaaaggcgtgctggccatgactgaagatgaaaccgtcgaagtgccaccggtgtgggtcgatgttgtcaacggcctcggcgctggcgatgccttcggtggcgcgctgtgccacggtctgttgtccgactggccactcgaaaaagtcctgcgctttgccaacgcggcaggctcggtggttgccggacgcttagagtgcagcaccgccatgccaaccactgaagaagttgaagcagccctaagtcagaaggtctag

SEQ ID NO: 2 - protein, 318 aa, synthetic construct
MAYLTSAHEVLAIGRLGVDIYPLQSGVGLEEVSSFGKYLGGSAANVSVAAARHGHNSALLSRVGNDPLGKYLLNELERLGVDNQYVATDPTYKTPLTLCEIFPPDDFPLYFYREPKAPDMCIESSDVNLEDVRDAEILWFTLTGLNEEPSRGAHQEILNTRARRKHTILDLDYRDMFWNSKQEATEQAQWALEHATVAVGNKEECEVAIGETEPERAGKALLEHGVKLAIVKQGPKGVLAMTEDETVEVPPVWVDVVNGLGAGDAFGGALCHGLLSDWPLEKVLRFANAAGSVVAGRLECSTAMPTTEEVEAALSQKV

SEQ ID NO: 3 - DNA, 957 bp, Corynebacterium stationis
  source 1..957: mol_type = genomic DNA
atggcgtatttaactagcgctcacgaagttctggccatcggcaggcttggcgtggatatctatccactacagtccggcgttgggctagaagaggtatcttctttcggcaaatacctaggcggatccgcagcaaatgtctctgttgcagccgcacggcacgggcacaattccgcactgctatcacgagtaggcaatgacccactgggtaagtacctgctcaatgagctggaaaggctcggggtagataatcagtacgtcgctactgatccgacttataaaaccccgctgactttgtgcgaaattttcccaccagatgatttcccgctgtacttctaccgcgagcccaaagctccggatatgtgcatcgagtcctctgacgtcaacctcgaagatgtccgcgatgcagaaatcttgtggtttaccctgaccggtttaagcgaagagccaagccgcggcgcacatcaggaaatcctgaacacccgcgcccggcgcaagcacaccatcttggacttggactaccgcgacatgttctggaattccaagcaggaagcaacagagcaggcacagtgggcactcgagcatgccaccgttgcggtcggtaacaaggaagaatgcgaggtcgccatcggcgaaaccgaaccagaacgcgccggcaaggcgttgttggaacatggcgtgaagttggccatcgttaagcaaggccccaaaggcgtgctggccatgactgaagatgaaaccgtcgaagtgccaccggtgtgggtcgatgttgtcaacggcctcggcgctggcgatgccttcggtggcgcgctgtgccacggtctgttgtccgactggccactcgaaaaagtcctgcgctttgccaacgcggcaggctcggtggttgccggacgcttagagtgcagcaccgccatgccaaccactgaagaagttgaagcagccctaagtcagaaggtctag

SEQ ID NO: 4 - protein, 318 aa, Corynebacterium stationis
MAYLTSAHEVLAIGRLGVDIYPLQSGVGLEEVSSFGKYLGGSAANVSVAAARHGHNSALLSRVGNDPLGKYLLNELERLGVDNQYVATDPTYKTPLTLCEIFPPDDFPLYFYREPKAPDMCIESSDVNLEDVRDAEILWFTLTGLSEEPSRGAHQEILNTRARRKHTILDLDYRDMFWNSKQEATEQAQWALEHATVAVGNKEECEVAIGETEPERAGKALLEHGVKLAIVKQGPKGVLAMTEDETVEVPPVWVDVVNGLGAGDAFGGALCHGLLSDWPLEKVLRFANAAGSVVAGRLECSTAMPTTEEVEAALSQKV

SEQ ID NO: 5 - DNA, 5719 bp, synthetic construct
  source 1..5719: mol_type = other DNA
tgccgcaagcactcagggcgcaagggctgctaaaggaagcggaacacgtagaaagccagtccgcagaaacggtgctgaccccggatgaatgtcagctactgggctatctggacaagggaaaacgcaagcgcaaagagaaagcaggtagcttgcagtgggcttacatggcgatagctagactgggcggttttatggacagcaagcgaaccggaattgccagctggggcgccctctggtaaggttgggaagccctgcaaagtaaactggatggctttcttgccgccaaggatctgatggcgcaggggatcaagatctgatcaagagacaggatgaggatcgtttcgcatgattgaacaagatggattgcacgcaggttctccggccgcttgggtggagaggctattcggctatgactgggcacaacagacaatcggctgctctgatgccgccgtgttccggctgtcagcgcaggggcgcccggttctttttgtcaagaccgacctgtccggtgccctgaatgaactccaagacgaggcagcgcggctatcgtggctggccacgacgggcgttccttgcgcagctgtgctcgacgttgtcactgaagcgggaagggactggctgctattgggcgaagtgccggggcaggatctcctgtcatctcaccttgctcctgccgagaaagtatccatcatggctgatgcaatgcggcggctgcatacgcttgatccggctacctgcccattcgaccaccaagcgaaacatcgcatcgagcgagcacgtactcggatggaagccggtcttgtcgatcaggatgatctggacgaagagcatcaggggctcgcgccagccgaactgttcgccaggctcaaggcgcggatgcccgacggcgaggatctcgtcgtgacccatggcgatgcctgcttgccgaatatcatggtggaaaatggccgcttttctggattcatcgactgtggccggctgggtgtggcggaccgctatcaggacatagcgttggctacccgtgatattgctgaagagcttggcggcgaatgggctgaccgcttcctcgtgctttacggtatcgccgctcccgattcgcagcgcatcgccttctatcgccttcttgacgagttcttctgagcgggactctggggttcgctagaggatcgatcctttttaacccatcacatatacctgccgttcactattatttagtgaaatgagatattatgatattttctgaattgtgattaaaaaggcaactttatgcccatgcaacagaaactataaaaaatacagagaatgaaaagaaacagatagattttttagttctttaggcccgtagtctgcaaatccttttatgattttctatcaaacaaaagaggaaaatagaccagttgcaatccaaacgagagtctaatagaatgaggtcgaaaagtaaatcgcgcgggtttgttactgataaagcaggcaagacctaaaatgtgtaaagggcaaagtgtatactttggcgtcaccccttacatattttaggtctttttttattgtgcgtaactaacttgccatcttcaaacaggagggctggaagaagcagaccgctaacacagtacataaaaaaggagacatgaacgatgaacatcaaaaagtttgcaaaacaagcaacagtattaacctttactaccgcactgctggcaggaggcgcaactcaagcgtttgcgaaagaaacgaaccaaaagccatataaggaaacatacggcatttcccatattacacgccatgatatgctgcaaatccctgaacagcaaaaaaatgaaaaatatcaagtttctgaatttgattcgtccacaattaaaaatatctcttctgcaaaaggcctggacgtttgggacagctggccattacaaaacgctgacggcactgtcgcaaactatcacggctaccacatcgtctttgcattagccggagatcctaaaaatgcggatgacacatcgatttacatgttctatcaaaaagtcggcgaaacttctattgacagctggaaaaacgctggccgcgtctttaaagacagcgacaaattcgatgcaaatgattctatcctaaaagaccaaacacaagaatggtcaggttcagccacatttacatctgacggaaaaatccgtttattctacactgatttctccggtaaacattacggcaaacaaacactgacaactgcacaagttaacgtatcagcatcagacagctctttgaacatcaacggtgtagaggattataaatcaatctttgacggtgacggaaaaacgtatcaaaatgtacagcagttcatcgatgaaggcaactacagctcaggcgacaaccatacgctgagagatcctcactacgtagaagataaaggccacaaatacttagtatttgaagcaaacactggaactgaagatggctaccaaggcgaagaatctttatttaacaaagcatactatggcaaaagcacatcattcttccgtcaagaaagtcaaaaacttctgcaaagcgataaaaaacgcacggctgagttagcaaacggcgctctcggtatgattgagctaaacgatgattacacactgaaaaaagtgatgaaaccgctgattgcatctaacacagtaacagatgaaattgaacgcgcgaacgtctttaaaatgaacggcaaatggtacctgttcactgactcccgcggatcaaaaatgacgattgacggcattacgtctaacgatatttacatgcttggttatgtttctaattctttaactggcccatacaagccgctgaacaaaactggccttgtgttaaaaatggatcttgatcctaacgatgtaacctttacttactcacacttcgctgtacctcaagcgaaaggaaacaatgtcgtgattacaagctatatgacaaacagaggattctacgcagacaaacaatcaacgtttgcgccgagcttcctgctgaacatcaaaggcaagaaaacatctgttgtcaaagacagcatccttgaacaaggacaattaacagttaacaaataaaaacgcaaaagaaaatgccgatgggtaccgagcgaaatgaccgaccaagcgacgcccaacctgccatcacgagatttcgattccaccgccgccttctatgaaaggttgggcttcggaatcgttttccgggacgccctcgcggacgtgctcatagtccacgacgcccgtgattttgtagccctggccgacggccagcaggtaggccgacaggctcatgccggccgccgccgccttttcctcaatcgctcttcgttcgtctggaaggcagtacaccttgataggtgggctgcccttcctggttggcttggtttcatcagccatccgcttgccctcatctgttacgccggcggtagccggccagcctcgcagagcaggattcccgttgagcaccgccaggtgcgaataagggacagtgaagaaggaacacccgctcgcgggtgggcctacttcacctatcctgcccggctgacgccgttggatacaccaaggaaagtctacacgaaccctttggcaaaatcctgtatatcgtgcgaaaaaggatggatataccgaaaaaatcgctataatgaccccgaagcagggttatgcagcggaaaagcgctgcttccctgctgttttgtggaatatctaccgactggaaacaggcaaatgcaggaaattactgaactgaggggacaggcgagagacgatgccaaagagctcctgaaaatctcgataactcaaaaaatacgcccggtagtgatcttatttcattatggtgaaagttggaacctcttacgtgccgatcaacgtctcattttcgccaaaagttggcccagggcttcccggtatcaacagggacaccaggatttatttattctgcgaagtgatcttccgtcacaggtatttattcggcgcaaagtgcgtcgggtgatgctgccaacttactgatttagtgtatgatggtgtttttgaggtgctccagtggcttctgtttctatcagctcctgaaaatctcgataactcaaaaaatacgcccggtagtgatcttatttcattatggtgaaagttggaacctcttacgtgccgatcaacgtctcattttcgccaaaagttggcccagggcttcccggtatcaacagggacaccaggatttatttattctgcgaagtgatcttccgtcacaggtatttattcggcgcaaagtgcgtcgggtgatgctgccaacttactgatttagtgtatgatggtgtttttgaggtgctccagtggcttctgtttctatcagggctggatgatcctccagcgcggggatctcatgctggagttcttcgcccaccccaaaaggatctaggtgaagatcctttttgataatctcatgaccaaaatcccttaacgtgagttttcgttccactgagcgtcagaccccgtagaaaagatcaaaggatcttcttgagatcctttttttctgcgcgtaatctgctgcttgcaaacaaaaaaaccaccgctaccagcggtggtttgtttgccggatcaagagctaccaactctttttccgaaggtaactggcttcagcagagcgcagataccaaatactgttcttctagtgtagccgtagttaggccaccacttcaagaactctgtagcaccgcctacatacctcgctctgctaatcctgttaccagtggctgctgccagtggcgataagtcgtgtcttaccgggttggactcaagacgatagttaccggataaggcgcagcggtcgggctgaacggggggttcgtgcacacagcccagcttggagcgaacgacctacaccgaactgagatacctacagcgtgagctatgagaaagcgccacgcttcccgaagggagaaaggcggacaggtatccggtaagcggcagggtcggaacaggagagcgcacgagggagcttccagggggaaacgcctggtatctttatagtcctgtcgggtttcgccacctctgacttgagcgtcgatttttgtgatgctcgtcaggggggcggagcctatggaaaaacgccagcaacgcggcctttttacggttcctggccttttgctggccttttgctcacatgttctttcctgcgttatcccctgattctgtggataaccgtattaccgcctttgagtgagctgataccgctcgccgcagccgaacgaccgagcgcagcgagtcagtgagcgaggaagcggaagagcgcccaatacgcaaaccgcctctccccgcgcgttggccgattcattaatgcagctggcacgacaggtttcccgactggaaagcgggcagtgagcgcaacgcaattaatgtgagttagctcactcattaggcaccccaggctttacactttatgcttccggctcgtatgttgtgtggaattgtgagcggataacaatttcacacaggaaacagctatgacatgattacgccaagcttgcatgcctgcaggtcgactctagaggatccccgggtaccgagctcgaattcactggccgtcgttttacaacgtcgtgactgggaaaaccctggcgttacccaacttaatcgccttgcagcacatccccctttcgccagctggcgtaatagcgaagaggcccgcaccgatcgcccttcccaacagttgcgcagcctgaatggcgaatggcgataagctagcttcacgc

SEQ ID NO: 6 - DNA, 23 bp, synthetic construct
  source 1..23: mol_type = other DNA
aatgtgctattgtcaggacatgc

SEQ ID NO: 7 - DNA, 22 bp, synthetic construct
  source 1..22: mol_type = other DNA
ggctcttcgtttaaaccggtca

SEQ ID NO: 8 - DNA, 22 bp, synthetic construct
  source 1..22: mol_type = other DNA
tgaccggtttaaacgaagagcc

SEQ ID NO: 9 - DNA, 22 bp, synthetic construct
  source 1..22: mol_type = other DNA
accttctgacttagggctgctt